European Patent Specification EP 3 916 099 B1, published April 12, 2023. Title: Genome Engineering. Applicant: Church, George Yang, Luhan Cargol, Marc Yang, Joyce. Application PCT/US14/048140. The sequence listing filed with the application follows.

SEQUENCE LISTING (224 sequences)

SEQ ID NO: 1 - DNA, 15 bp, Artificial
  Oligonucleotide sequence
tggggcaagcttctg

SEQ ID NO: 2 - DNA, 102 bp, Artificial
  TALE template
  misc_feature (34)..(39): n is a, c, g, or t
ctaaccccagagcaggtcgtggcaatcgcctccnnnnnnggcggaaaacaggcattggaaacagtacagcggctgctgccggtgctgtgccaagcgcacgga

SEQ ID NO: 3 - DNA, 102 bp, Artificial
  PCR primer
  misc_feature (34)..(39): n is a, c, g, or t
ctaacccctgaacaggtagtcgctatagcttcannnnnngggggcaagcaagcacttgagaccgttcaacgactcctgccagtgctctgccaagcccatgga

SEQ ID NO: 4 - DNA, 102 bp, Artificial
  PCR primer
  misc_feature (34)..(39): n is a, c, g, or t
ttgactccggagcaagtcgtcgcgatcgcgagcnnnnnnggggggaagcaggcgctggaaactgttcagagactgctgcctgtactttgtcaggcgcatggt

SEQ ID NO: 5 - DNA, 102 bp, Artificial
  PCR primer
  misc_feature (34)..(39): n is a, c, g, or t
ctcacccccgaacaggttgtcgcaatagcaagtnnnnnnggcggtaagcaagccctagagactgtgcaacgcctgctccccgtgctgtgtcaggctcacggt

SEQ ID NO: 6 - DNA, 102 bp, Artificial
  PCR primer
  misc_feature (34)..(39): n is a, c, g, or t
ctgacacctgaacaagttgtcgcgatagccagtnnnnnngggggaaaacaagctctagaaacggttcaaaggttgttgcccgttctgtgccaagcacatggg

SEQ ID NO: 7 - DNA, 102 bp, Artificial
  PCR primer
  misc_feature (34)..(39): n is a, c, g, or t
ttaacacccgaacaagtagtagcgatagcgtcannnnnngggggtaaacaggctttggagacggtacagcggttattgccggtcctctgccaggcccacgga

SEQ ID NO: 8 - DNA, 102 bp, Artificial
  PCR primer
  misc_feature (34)..(39): n is a, c, g, or t
cttacgccagaacaggtggttgcaattgcctccnnnnnnggcgggaaacaagcgttggaaactgtgcagagactccttcctgttttgtgtcaagcccacggc

SEQ ID NO: 9 - DNA, 102 bp, Artificial
  PCR primer
  misc_feature (34)..(39): n is a, c, g, or t
ttgacgcctgagcaggttgtggccatcgctagcnnnnnnggagggaagcaggctcttgaaaccgtacagcgacttctcccagttttgtgccaagctcacggg

SEQ ID NO: 10 - DNA, 102 bp, Artificial
  PCR primer
  misc_feature (34)..(39): n is a, c, g, or t
ctaacccccgagcaagtagttgccatagcaagcnnnnnnggaggaaaacaggcattagaaacagttcagcgcttgctcccggtactctgtcaggcacacggt

SEQ ID NO: 11 - DNA, 102 bp, Artificial
  PCR primer
  misc_feature (34)..(39): n is a, c, g, or t
ctaactccggaacaggtcgtagccattgcttccnnnnnnggcggcaaacaggcgctagagacagtccagaggctcttgcctgtgttatgccaggcacatggc

SEQ ID NO: 12 - DNA, 102 bp, Artificial
  PCR primer
  misc_feature (34)..(39): n is a, c, g, or t
ctcaccccggagcaggtcgttgccatcgccagtnnnnnnggcggaaagcaagctctcgaaacagtacaacggctgttgccagtcctatgtcaagctcatgga

SEQ ID NO: 13 - DNA, 102 bp, Artificial
  PCR primer
  misc_feature (34)..(39): n is a, c, g, or t
ctgacgcccgagcaggtagtggcaatcgcatctnnnnnnggaggtaaacaagcactcgagactgtccaaagattgttacccgtactatgccaagcgcatggt

SEQ ID NO: 14 - DNA, 102 bp, Artificial
  PCR primer
  misc_feature (34)..(39): n is a, c, g, or t
ttaaccccagagcaagttgtggctattgcatctnnnnnnggtggcaaacaagccttggagacagtgcaacgattactgcctgtcttatgtcaggcccatggc

SEQ ID NO: 15 - DNA, 102 bp, Artificial
  PCR primer
  misc_feature (34)..(39): n is a, c, g, or t
cttactcctgagcaagtcgtagctatcgccagcnnnnnnggtgggaaacaggccctggaaaccgtacaacgtctcctcccagtactttgtcaagcacacggg

SEQ ID NO: 16 - DNA, 102 bp, Artificial
  PCR primer
  misc_feature (34)..(39): n is a, c, g, or t
ttgacaccggaacaagtggtggcgattgcgtccnnnnnnggaggcaagcaggcactggagaccgtccaacggcttcttccggttctttgccaggctcatggg

SEQ ID NO: 17 - DNA, 102 bp, Artificial
  PCR primer
  misc_feature (34)..(39): n is a, c, g, or t
ctcacgccagagcaggtggtagcaatagcgtcgnnnnnnggtggtaagcaagcgcttgaaacggtccagcgtcttctgccggtgttgtgccaggcgcacgga

SEQ ID NO: 18 - DNA, 102 bp, Artificial
  PCR primer
  misc_feature (34)..(39): n is a, c, g, or t
ctcacaccagaacaagtggttgctattgctagtnnnnnnggtggaaagcaggccctcgagacggtgcagaggttacttcccgtcctctgtcaagcgcacggc

SEQ ID NO: 19 - DNA, 60 bp, Artificial
  PCR primer
  misc_feature (34)..(39): n is a, c, g, or t
ctcactccagagcaagtggttgcgatcgcttcannnnnnggtggaagacctgccctggaa

SEQ ID NO: 20 - DNA, 5714 bp, Artificial
  Oligonucleotide sequence encoding TALEN backbone
atgtcgcggacccggctcccttccccacccgcacccagcccagcgttttcggccgactcgttctcagacctgcttaggcagttcgacccctcactgtttaacacatcgttgttcgactcccttcctccgtttggggcgcaccatacggaggcggccaccggggagtgggatgaggtgcagtcgggattgagagctgcggatgcaccacccccaaccatgcgggtggccgtcaccgctgcccgaccgccgagggcgaagcccgcaccaaggcggagggcagcgcaaccgtccgacgcaagccccgcagcgcaagtagatttgagaactttgggatattcacagcagcagcaggaaaagatcaagcccaaagtgaggtcgacagtcgcgcagcatcacgaagcgctggtgggtcatgggtttacacatgcccacatcgtagccttgtcgcagcaccctgcagcccttggcacggtcgccgtcaagtaccaggacatgattgcggcgttgccggaagccacacatgaggcgatcgtcggtgtggggaaacagtggagcggagcccgagcgcttgaggccctgttgacggtcgcgggagagctgagagggcctccccttcagctggacacgggccagttgctgaagatcgcgaagcggggaggagtcacggcggtcgaggcggtgcacgcgtggcgcaatgcgctcacgggagcacccctcaacagttcacgctgacagagaccgcggccgcattaggcaccccaggctttacactttatgcttccggctcgtataatgtgtggattttgagttaggatccgtcgagattttcaggagctaaggaagctaaaatggagaaaaaaatcactggatataccaccgttgatatatcccaatggcatcgtaaagaacattttgaggcatttcagtcagttgctcaatgtacctataaccagaccgttcagctggatattacggcctttttaaagaccgtaaagaaaaataagcacaagttttatccggcctttattcacattcttgcccgcctgatgaatgctcatccggaattccgtatggcaatgaaagacggtgagctggtgatatgggatagtgttcacccttgttacaccgttttccatgagcaaactgaaacgttttcatcgctctggagtgaataccacgacgatttccggcagtttctacacatatattcgcaagatgtggcgtgttacggtgaaaacctggcctatttccctaaagggtttattgagaatatgtttttcgtctcagccaatccctgggtgagtttcaccagttttgatttaaacgtggccaatatggacaacttcttcgcccccgttttcaccatgggcaaatattatacgcaaggcgacaaggtgctgatgccgctggcgattcaggttcatcatgccgtttgtgatggcttccatgtcggcagaatgcttaatgaattacaacagtactgcgatgagtggcagggcggggcgtaaagatctggatccggcttactaaaagccagataacagtatgcgtatttgcgcgctgatttttgcggtataagaatatatactgatatgtatacccgaagtatgtcaaaaagaggtatgctatgaagcagcgtattacagtgacagttgacagcgacagctatcagttgctcaaggcatatatgatgtcaatatctccggtctggtaagcacaaccatgcagaatgaagcccgtcgtctgcgtgccgaacgctggaaagcggaaaatcaggaagggatggctgaggtcgcccggtttattgaaatgaacggctcttttgctgacgagaacaggggctggtgaaatgcagtttaaggtttacacctataaaagagagagccgttatcgtctgtttgtggatgtacagagtgatattattgacacgcccgggcgacggatggtgatccccctggccagtgcacgtctgctgtcagataaagtctcccgtgaactttacccggtggtgcatatcggggatgaaagctggcgcatgatgaccaccgatatggccagtgtgccggtctccgttatcggggaagaagtggctgatctcagccaccgcgaaaatgacatcaaaaacgccattaacctgatgttctggggaatataaatgtcaggctcccttatacacagccagtctgcaggtcgacggtctcgctcttcgaaggttacttcccgtcctctgtcaagcgcacggcctcactccagagcaagtggttgcgatcgcttcaaacaacggtggaagacctgccctggaatcaatcgtggcccagctttcgaggccggaccccgcgctggccgcactcactaatgatcatcttgtagcgctggcctgcctcggcggacgacccgccttggatgcggtgaagaaggggctcccgcacgcgcctgcattgattaagcggaccaacagaaggattcccgagaggacatcacatcgagtggcaggttcccaactcgtgaagagtgaacttgaggagaaaaagtcggagctgcggcacaaattgaaatacgtaccgcatgaatacatcgaacttatcgaaattgctaggaactcgactcaagacagaatccttgagatgaaggtaatggagttctttatgaaggtttatggataccgagggaagcatctcggtggatcacgaaaacccgacggagcaatctatacggtggggagcccgattgattacggagtgatcgtcgacacgaaagcctacagcggtgggtacaatcttcccatcgggcaggcagatgagatgcaacgttatgtcgaagaaaatcagaccaggaacaaacacatcaatccaaatgagtggtggaaagtgtatccttcatcagtgaccgagtttaagtttttgtttgtctctgggcatttcaaaggcaactataaggcccagctcacacggttgaatcacattacgaactgcaatggtgcggttttgtccgtagaggaactgctcattggtggagaaatgatcaaagcgggaactctgacactggaagaagtcagacgcaagtttaacaatggcgagatcaatttccgcaagctaaaatggagaaaaaaatcactggatataccaccgttgatatatcccaatggcatcgtaaagaacattttgaggcatttcagtcagttgctcaatgtacctataaccagaccgttcagctggatattacggcctttttaaagaccgtaaagaaaaataagcacaagttttatccggcctttattcacattcttgcccgcctgatgaatgctcatccggaattccgtatggcaatgaaagacggtgagctggtgatatgggatagtgttcacccttgttacaccgttttccatgagcaaactgaaacgttttcatcgctctggagtgaataccacgacgatttccggcagtttctacacatatattcgcaagatgtggcgtgttacggtgaaaacctggcctatttccctaaagggtttattgagaatatgtttttcgtctcagccaatccctgggtgagtttcaccagttttgatttaaacgtggccaatatggacaacttcttcgcccccgttttcaccatgggcaaatattatacgcaaggcgacaaggtgctgatgccgctggcgattcaggttcatcatgccgtttgtgatggcttccatgtcggcagaatgcttaatgaattacaacagtactgcgatgagtggcagggcggggcgtaaagatctggatccggcttactaaaagccagataacagtatgcgtatttgcgcgctgatttttgcggtataagaatatatactgatatgtatacccgaagtatgtcaaaaagaggtatgctatgaagcagcgtattacagtgacagttgacagcgacagctatcagttgctcaaggcatatatgatgtcaatatctccggtctggtaagcacaaccatgcagaatgaagcccgtcgtctgcgtgccgaacgctggaaagcggaaaatcaggaagggatggctgaggtcgcccggtttattgaaatgaacggctcttttgctgacgagaacaggggctggtgaaatgcagtttaaggtttacacctataaaagagagagccgttatcgtctgtttgtggatgtacagagtgatattattgacacgcccgggcgacggatggtgatccccctggccagtgcacgtctgctgtcagataaagtctcccgtgaactttacccggtggtgcatatcggggatgaaagctggcgcatgatgaccaccgatatggccagtgtgccggtctccgttatcggggaagaagtggctgatctcagccaccgcgaaaatgacatcaaaaacgccattaacctgatgttctggggaatataaatgtcaggctcccttatacacagccagtctgcaggtcgacggtctcgctcttcgaaggttacttcccgtcctctgtcaagcgcacggcctcactccagagcaagtggttgcgatcgcttcaaacaacggtggaagacctgccctggaatcaatcgtggcccagctttcgaggccggaccccgcgctggccgcactcactaatgatcatcttgtagcgctggcctgcctcggcggacgacccgccttggatgcggtgaagaaggggctcccgcacgcgcctgcattgattaagcggaccaacagaaggattcccgagaggacatagccccaagaagaagagaaaggtggaggccagcggttccggacgggctgacgcattggacgattttgatctggatatgctgggaagtgacgccctcgatgattttgaccttgacatgcttggttcggatgcccttgatgactttgacctcgacatgctcggcagtgacgcccttgatgatttcgacctggacatgctgattaactctagaggcagtggagagggcagaggaagtctgctaacatgcggtgacgtcgaggagaatcctggcccagtgagcaagggcgaggagctgttcaccggggtggtgcccatcctggtcgagctggacggcgacgtaaacggccacaagttcagcgtgtccggcgagggcgagggcgatgccacctacggcaagctgaccctgaagttcatctgcaccaccggcaagctgcccgtgccctggcccaccctcgtgaccaccctgacctacggcgtgcagtgcttcagccgctaccccgaccacatgaagcagcacgacttcttcaagtccgccatgcccgaaggctacgtccaggagcgcaccatcttcttcaaggacgacggcaactacaagacccgcgccgaggtgaagttcgagggcgacaccctggtgaaccgcatcgagctgaagggcatcgacttcaaggaggacggcaacatcctggggcacaagctggagtacaactacaacagccacaacgtctatatcatggccgacaagcagaagaacggcatcaaggtgaacttcaagatccgccacaacatcgaggacggcagcgtgcagctcgccgaccactaccagcagaacacccccatcggcgacggccccgtgctgctgcccgacaaccactacctgagcacccagtccgccctgagcaaagaccccaacgagaagcgcgatcacatggtcctgctggagttcgtgaccgccgccgggatcactctcggcatggacgagctgtacaag

SEQ ID NO: 21 - DNA, 3465 bp, Artificial
  Oligonucleotide sequence encoding TALE backbone sequence
atgtcgcggacccggctcccttccccacccgcacccagcccagcgttttcggccgactcgttctcagacctgcttaggcagttcgacccctcactgtttaacacatcgttgttcgactcccttcctccgtttggggcgcaccatacggaggcggccaccggggagtgggatgaggtgcagtcgggattgagagctgcggatgcaccacccccaaccatgcgggtggccgtcaccgctgcccgaccgccgagggcgaagcccgcaccaaggcggagggcagcgcaaccgtccgacgcaagccccgcagcgcaagtagatttgagaactttgggatattcacagcagcagcaggaaaagatcaagcccaaagtgaggtcgacagtcgcgcagcatcacgaagcgctggtgggtcatgggtttacacatgcccacatcgtagccttgtcgcagcaccctgcagcccttggcacggtcgccgtcaagtaccaggacatgattgcggcgttgccggaagccacacatgaggcgatcgtcggtgtggggaaacagtggagcggagcccgagcgcttgaggccctgttgacggtcgcgggagagctgagagggcctccccttcagctggacacgggccagttgctgaagatcgcgaagcggggaggagtcacggcggtcgaggcggtgcacgcgtggcgcaatgcgctcacgggagcacccctcaacagttcacgctgacagagaccgcggccgcattaggcaccccaggctttacactttatgcttccggctcgtataatgtgtggattttgagttaggatccgtcgagattttcaggagctaaggaagctaaaatggagaaaaaaatcactggatataccaccgttgatatatcccaatggcatcgtaaagaacattttgaggcatttcagtcagttgctcaatgtacctataaccagaccgttcagctggatattacggcctttttaaagaccgtaaagaaaaataagcacaagttttatccggcctttattcacattcttgcccgcctgatgaatgctcatccggaattccgtatggcaatgaaagacggtgagctggtgatatgggatagtgttcacccttgttacaccgttttccatgagcaaactgaaacgttttcatcgctctggagtgaataccacgacgatttccggcagtttctacacatatattcgcaagatgtggcgtgttacggtgaaaacctggcctatttccctaaagggtttattgagaatatgtttttcgtctcagccaatccctgggtgagtttcaccagttttgatttaaacgtggccaatatggacaacttcttcgcccccgttttcaccatgggcaaatattatacgcaaggcgacaaggtgctgatgccgctggcgattcaggttcatcatgccgtttgtgatggcttccatgtcggcagaatgcttaatgaattacaacagtactgcgatgagtggcagggcggggcgtaaagatctggatccggcttactaaaagccagataacagtatgcgtatttgcgcgctgatttttgcggtataagaatatatactgatatgtatacccgaagtatgtcaaaaagaggtatgctatgaagcagcgtattacagtgacagttgacagcgacagctatcagttgctcaaggcatatatgatgtcaatatctccggtctggtaagcacaaccatgcagaatgaagcccgtcgtctgcgtgccgaacgctggaaagcggaaaatcaggaagggatggctgaggtcgcccggtttattgaaatgaacggctcttttgctgacgagaacaggggctggtgaaatgcagtttaaggtttacacctataaaagagagagccgttatcgtctgtttgtggatgtacagagtgatattattgacacgcccgggcgacggatggtgatccccctggccagtgcacgtctgctgtcagataaagtctcccgtgaactttacccggtggtgcatatcggggatgaaagctggcgcatgatgaccaccgatatggccagtgtgccggtctccgttatcggggaagaagtggctgatctcagccaccgcgaaaatgacatcaaaaacgccattaacctgatgttctggggaatataaatgtcaggctcccttatacacagccagtctgcaggtcgacggtctcgctcttcgaaggttacttcccgtcctctgtcaagcgcacggcctcactccagagcaagtggttgcgatcgcttcaaacaacggtggaagacctgccctggaatcaatcgtggcccagctttcgaggccggaccccgcgctggccgcactcactaatgatcatcttgtagcgctggcctgcctcggcggacgacccgccttggatgcggtgaagaaggggctcccgcacgcgcctgcattgattaagcggaccaacagaaggattcccgagaggacatagccccaagaagaagagaaaggtggaggccagcggttccggacgggctgacgcattggacgattttgatctggatatgctgggaagtgacgccctcgatgattttgaccttgacatgcttggttcggatgcccttgatgactttgacctcgacatgctcggcagtgacgcccttgatgatttcgacctggacatgctgattaactctagaggcagtggagagggcagaggaagtctgctaacatgcggtgacgtcgaggagaatcctggcccagtgagcaagggcgaggagctgttcaccggggtggtgcccatcctggtcgagctggacggcgacgtaaacggccacaagttcagcgtgtccggcgagggcgagggcgatgccacctacggcaagctgaccctgaagttcatctgcaccaccggcaagctgcccgtgccctggcccaccctcgtgaccaccctgacctacggcgtgcagtgcttcagccgctaccccgaccacatgaagcagcacgacttcttcaagtccgccatgcccgaaggctacgtccaggagcgcaccatcttcttcaaggacgacggcaactacaagacccgcgccgaggtgaagttcgagggcgacaccctggtgaaccgcatcgagctgaagggcatcgacttcaaggaggacggcaacatcctggggcacaagctggagtacaactacaacagccacaacgtctatatcatggccgacaagcagaagaacggcatcaaggtgaacttcaagatccgccacaacatcgaggacggcagcgtgcagctcgccgaccactaccagcagaacacccccatcggcgacggccccgtgctgctgcccgacaaccactacctgagcacccagtccgccctgagcaaagaccccaacgagaagcgcgatcacatggtcctgctggagttcgtgaccgccgccgggatcactctcggcatggacgagctgtacaag

SEQ ID NO: 22 - protein, 1368 aa, Streptococcus pyogenes [sequence omitted]

SEQ ID NO: 23 - DNA, 82 bp, Artificial
  Oligonucleotide sequence
  misc_feature (41)..(41): n is a, c, g, or t
ttcttggctttatatatcttgtggaaaggacgaaacaccgngttttagagctagaaatagcaagttaaaataaggctagtcc

SEQ ID NO: 24 - DNA, 1692 bp, Artificial
  Oligonucleotide sequence encoding re-TALE
ctaacccctgaacaggtagtcgctatagcttcaaatatcgggggcaagcaagcacttgagaccgttcaacgactcctgccagtgctctgccaagcccatggattgactccggagcaagtcgtcgcgatcgcgagcaacggcggggggaagcaggcgctggaaactgttcagagactgctgcctgtactttgtcaggcgcatggtctcacccccgaacaggttgtcgcaatagcaagtaatataggcggtaagcaagccctagagactgtgcaacgcctgctccccgtgctgtgtcaggctcacggtctgacacctgaacaagttgtcgcgatagccagtcacgacgggggaaaacaagctctagaaacggttcaaaggttgttgcccgttctgtgccaagcacatgggttaacacccgaacaagtagtagcgatagcgtcaaataacgggggtaaacaggctttggagacggtacagcggttattgccggtcctctgccaggcccacggacttacgccagaacaggtggttgcaattgcctccaacatcggcgggaaacaagcgttggaaactgtgcagagactccttcctgttttgtgtcaagcccacggcttgacgcctgagcaggttgtggccatcgctagccacgacggagggaagcaggctcttgaaaccgtacagcgacttctcccagttttgtgccaagctcacgggctaacccccgagcaagtagttgccatagcaagcaacggaggaggaaaacaggcattagaaacagttcagcgcttgctcccggtactctgtcaggcacacggtctaactccggaacaggtcgtagccattgcttcccatgatggcggcaaacaggcgctagagacagtccagaggctcttgcctgtgttatgccaggcacatggcctcaccccggagcaggtcgttgccatcgccagtaatatcggcggaaagcaagctctcgaaacagtacaacggctgttgccagtcctatgtcaagctcatggactgacgcccgagcaggtagtggcaatcgcatctcacgatggaggtaaacaagcactcgagactgtccaaagattgttacccgtactatgccaagcgcatggtttaaccccagagcaagttgtggctattgcatctaacggcggtggcaaacaagccttggagacagtgcaacgattactgcctgtcttatgtcaggcccatggccttactcctgagcaagtcgtagctatcgccagcaacataggtgggaaacaggccctggaaaccgtacaacgtctcctcccagtactttgtcaagcacacgggttgacaccggaacaagtggtggcgattgcgtccaacggcggaggcaagcaggcactggagaccgtccaacggcttcttccggttctttgccaggctcatgggctcacgccagagcaggtggtagcaatagcgtcgaacatcggtggtaagcaagcgcttgaaacggtccagcgtcttctgccggtgttgtgccaggcgcacggactcacaccagaacaagtggttgctattgctagtaacaacggtggaaagcaggccctcgagacggtgcagaggttacttcccgtcctctgtcaagcgcacggcctcactccagagcaagtggttgcgatcgcttcaaacaatggtggaagacctgccctggaa

SEQ ID NO: 25 - DNA, 237 bp, Artificial
  Template sequence
  misc_feature (64)..(69): n is a, c, g, or t
  misc_feature (166)..(171): n is a, c, g, or t
cgcaatgcgctcacgggagcacccctcaacctaacccctgaacaggtagtcgctatagcttcannnnnngggggcaagcaagcacttgagaccgttcaacgactcctgccagtgctctgccaagcccatggattgactccggagcaagtcgtcgcgatcgcgagcnnnnnnggggggaagcaggcgctggaaactgttcagagactgctgcctgtactttgtcaggcgcatggtctc

SEQ ID NO: 26 - DNA, 240 bp, Artificial
  Template sequence
  misc_feature (67)..(72): n is a, c, g, or t
  misc_feature (169)..(174): n is a, c, g, or t
agactgctgcctgtactttgtcaggcgcatggtctcacccccgaacaggttgtcgcaatagcaagtnnnnnnggcggtaagcaagccctagagactgtgcaacgcctgctccccgtgctgtgtcaggctcacggtctgacacctgaacaagttgtcgcgatagccagtnnnnnngggggaaaacaagctctagaaacggttcaaaggttgttgcccgttctgtgccaagcacatgggtta

SEQ ID NO: 27 - DNA, 232 bp, Artificial
  Template sequence
  misc_feature (59)..(64): n is a, c, g, or t
  misc_feature (161)..(166): n is a, c, g, or t
tgcgctcacgggagcacccctcaacctcacccccgaacaggttgtcgcaatagcaagtnnnnnnggcggtaagcaagccctagagactgtgcaacgcctgctccccgtgctgtgtcaggctcacggtctgacacctgaacaagttgtcgcgatagccagtnnnnnngggggaaaacaagctctagaaacggttcaaaggttgttgcccgttctgtgccaagcacatgggtta

SEQ ID NO: 28 - DNA, 246 bp, Artificial
  Template sequence
  misc_feature (67)..(72): n is a, c, g, or t
  misc_feature (169)..(174): n is a, c, g, or t
aggttgttgcccgttctgtgccaagcacatgggttaacacccgaacaagtagtagcgatagcgtcannnnnngggggtaaacaggctttggagacggtacagcggttattgccggtcctctgccaggcccacggacttacgccagaacaggtggttgcaattgcctccnnnnnnggcgggaaacaagcgttggaaactgtgcagagactccttcctgttttgtgtcaagcccacggcttgacgcct

SEQ ID NO: 29 - DNA, 240 bp, Artificial
  Template sequence
  misc_feature (67)..(72): n is a, c, g, or t
  misc_feature (169)..(174): n is a, c, g, or t
agactccttcctgttttgtgtcaagcccacggcttgacgcctgagcaggttgtggccatcgctagcnnnnnnggagggaagcaggctcttgaaaccgtacagcgacttctcccagttttgtgccaagctcacgggctaacccccgagcaagtagttgccatagcaagcnnnnnnggaggaaaacaggcattagaaacagttcagcgcttgctcccggtactctgtcaggcacacggtcta

SEQ ID NO: 30 - DNA, 240 bp, Artificial
  Template sequence
  misc_feature (67)..(72): n is a, c, g, or t
  misc_feature (169)..(174): n is a, c, g, or t
cgcttgctcccggtactctgtcaggcacacggtctaactccggaacaggtcgtagccattgcttccnnnnnnggcggcaaacaggcgctagagaccgtccagaggctcttgcctgtgttatgccaggcacatggcctcaccccggagcaggtcgttgccatcgccagtnnnnnnggcggaaagcaagctctcgaaacagtacaacggctgttgccagtcctatgtcaagctcatggactg

SEQ ID NO: 31 - DNA, 240 bp, Artificial
  Template sequence
  misc_feature (67)..(72): n is a, c, g, or t
  misc_feature (169)..(174): n is a, c, g, or t
cggctgttgccagtcctatgtcaagctcatggactgacgcccgagcaggtagtggcaatcgcatctnnnnnnggaggtaaacaagcactcgagactgtccaaagattgttacccgtactatgccaagcgcatggtttaaccccagagcaagttgtggctattgcatctnnnnnnggtggcaaacaagccttggagaccgtgcaacgattactgcctgtcttatgtcaggcccatggcctt

SEQ ID NO: 32 - DNA, 240 bp, Artificial
  Template sequence
  misc_feature (67)..(72): n is a, c, g, or t
  misc_feature (169)..(174): n is a, c, g, or t
cgattactgcctgtcttatgtcaggcccatggccttactcctgagcaggtggtcgctatcgccagcnnnnnngggggcaagcaagcactggaaacagtccagcgtttgcttccagtactttgtcaggcgcatggattgacaccggaacaagtggtggctatagcctcannnnnnggaggaaagcaggcgctggaaaccgtccaacgtcttttaccggtgctttgccaggcgcacgggctc

SEQ ID NO: 33 - DNA, 240 bp, Artificial
  Template sequence
  misc_feature (67)..(72): n is a, c, g, or t
  misc_feature (169)..(174): n is a, c, g, or t
cgattactgcctgtcttatgtcaggcccatggccttactcctgagcaagtcgtagctatcgccagcnnnnnnggtgggaaacaggccctggaaaccgtacaacgtctcctcccagtactttgtcaagcacacgggttgacaccggaacaagtggtggcgattgcgtccnnnnnnggaggcaagcaggcactggagaccgtccaacggcttcttccggttctttgccaggctcatgggctc

SEQ ID NO: 34 - DNA, 240 bp, Artificial
  Template sequence
  misc_feature (67)..(72): n is a, c, g, or t
  misc_feature (169)..(174): n is a, c, g, or t
cggcttcttccggttctttgccaggctcatgggctcacgccagagcaggtggtagcaatagcgtcgnnnnnnggtggtaagcaagcgcttgaaacggtccagcgtcttctgccggtgttgtgccaggcgcacggactcacaccagaacaagtggttgctattgctagtnnnnnnggtggaaagcaggccctcgagacggtgcagaggttacttcccgtcctctgtcaagcgcacggcctc

SEQ ID NO: 35 - DNA, 49 bp, Artificial
  Primer sequence
cgcaatgcgctcacgggagcacccctcaacctaacccctgaacaggtag

SEQ ID NO: 36 - DNA, 46 bp, Artificial
  Primer sequence
gagaccatgcgcctgacaaagtacaggcagcagtctctgaacagtt

SEQ ID NO: 37 - DNA, 33 bp, Artificial
  Primer sequence
tggcgcaatgcgctcacgggagcacccctcaac

SEQ ID NO: 38 - DNA, 49 bp, Artificial
  Primer sequence
agactgctgcctgtactttgtcaggcgcatggtctcacccccgaacagg

SEQ ID NO: 39 - DNA, 46 bp, Artificial
  Primer sequence
taacccatgtgcttggcacagaacgggcaacaacctttgaaccgtt

SEQ ID NO: 40 - DNA, 48 bp, Artificial
  Primer sequence
aggttgttgcccgttctgtgccaagcacatgggttaacacccgaacaa

SEQ ID NO: 41 - DNA, 52 bp, Artificial
  Primer sequence
aggcgtcaagccgtgggcttgacacaaaacaggaaggagtctctgcacagtt

SEQ ID NO: 42 - DNA, 45 bp, Artificial
  Primer sequence
agactccttcctgttttgtgtcaagcccacggcttgacgcctgag

SEQ ID NO: 43 - DNA, 40 bp, Artificial
  Primer sequence
tagaccgtgtgcctgacagagtaccgggagcaagcgctga

SEQ ID NO: 44 - DNA, 39 bp, Artificial
  Primer sequence
cgcttgctcccggtactctgtcaggcacacggtctaact

SEQ ID NO: 45 - DNA, 40 bp, Artificial
  Primer sequence
cagtccatgagcttgacataggactggcaacagccgttgt

SEQ ID NO: 46 - DNA, 39 bp, Artificial
  Primer sequence
cggctgttgccagtcctatgtcaagctcatggactgacg

SEQ ID NO: 47 - DNA, 40 bp, Artificial
  Primer sequence
aaggccatgggcctgacataagacaggcagtaatcgttgc

SEQ ID NO: 48 - DNA, 39 bp, Artificial
  Primer sequence
cgattactgcctgtcttatgtcaggcccatggccttact

SEQ ID NO: 49 - DNA, 43 bp, Artificial
  Primer sequence
gagcccgtgcgcctggcaaagcaccggtaaaagacgttggacg

SEQ ID NO: 50 - DNA, 50 bp, Artificial
  Primer sequence
cgattactgcctgtcttatgtcaggcccatggccttactcctgagcaagt

SEQ ID NO: 51 - DNA, 40 bp, Artificial
  Primer sequence
gagcccatgagcctggcaaagaaccggaagaagccgttgg

SEQ ID NO: 52 - DNA, 51 bp, Artificial
  Primer sequence
cggcttcttccggttctttgccaggctcatgggctcacgccagagcaggtg

SEQ ID NO: 53 - DNA, 40 bp, Artificial
  Primer sequence
gaggccgtgcgcttgacagaggacgggaagtaacctctgc

SEQ ID NO: 54 - DNA, 18 bp, Artificial
  Targeting sequence
tccccactttcttgtgaa

SEQ ID NO: 55 - DNA, 18 bp, Artificial
  Targeting sequence
taaccactcaggacaggg

SEQ ID NO: 56 - DNA, 19 bp, Artificial
  Targeting sequence
cactttcttgtgaatcctt

SEQ ID NO: 57 - DNA, 18 bp, Artificial
  Targeting sequence
tcacacagcaagtcagca

SEQ ID NO: 58 - DNA, 18 bp, Artificial
  Targeting sequence
tagcggagcaggctcgga

SEQ ID NO: 59 - DNA, 19 bp, Artificial
  Targeting sequence
tgggctagcggagcaggct

SEQ ID NO: 60 - DNA, 18 bp, Artificial
  Targeting sequence
tacccagacgagaaagct

SEQ ID NO: 61 - DNA, 18 bp, Artificial
  Targeting sequence
tcagactgccaagcttga

SEQ ID NO: 62 - DNA, 19 bp, Artificial
  Targeting sequence
acccagacgagaaagctga

SEQ ID NO: 63 - DNA, 18 bp, Artificial
  Targeting sequence
tcttgtggctcgggagta

SEQ ID NO: 64 - DNA, 18 bp, Artificial
  Targeting sequence
tattgtcagcagagctga

SEQ ID NO: 65 - DNA, 19 bp, Artificial
  Targeting sequence
agagggcatcttgtggctc

SEQ ID NO: 66 - DNA, 18 bp, Artificial
  Targeting sequence
ttgagattttcagatgtc

SEQ ID NO: 67 - DNA, 18 bp, Artificial
  Targeting sequence
tatacagtcatatcaagc

SEQ ID NO: 68 - DNA, 19 bp, Artificial
  Targeting sequence
atcaagctctcttggcggt

SEQ ID NO: 69 - DNA, 18 bp, Artificial
  Targeting sequence
ttcagatagattatatct

SEQ ID NO: 70 - DNA, 18 bp, Artificial
  Targeting sequence
tgccagatacataggtgg

SEQ ID NO: 71 - DNA, 19 bp, Artificial
  Targeting sequence
gcttcagatagattatatc

SEQ ID NO: 72 - DNA, 18 bp, Artificial
  Targeting sequence
ttatactgtctatatgat

SEQ ID NO: 73 - DNA, 18 bp, Artificial
  Targeting sequence
tcagctcttctggccaga

SEQ ID NO: 74 - DNA, 19 bp, Artificial
  Targeting sequence
acggatgtctcagctcttc

SEQ ID NO: 75 - DNA, 18 bp, Artificial
  Targeting sequence
tggccagaagagctgaga

SEQ ID NO: 76 - DNA, 18 bp, Artificial
  Targeting sequence
ttaccggggagagtttct

SEQ ID NO: 77 - DNA, 19 bp, Artificial
  Targeting sequence
ccggggagagtttcttgta

SEQ ID NO: 78 - DNA, 18 bp, Artificial
  Targeting sequence
tttgcagagagatgagtc

SEQ ID NO: 79 - DNA, 18 bp, Artificial
  Targeting sequence
ttagcagaagataagatt

SEQ ID NO: 80 - DNA, 19 bp, Artificial
  Targeting sequence
gaaatcttatcttctgcta

SEQ ID NO: 81 - DNA, 18 bp, Artificial
  Targeting sequence
tataagactaaactaccc

SEQ ID NO: 82 - DNA, 18 bp, Artificial
  Targeting sequence
tcgtctgccaccacagat

SEQ ID NO: 83 - DNA, 19 bp, Artificial
  Targeting sequence
aatgcatgacattcatctg

SEQ ID NO: 84 - DNA, 18 bp, Artificial
  Targeting sequence
taaaacagtttgcattca

SEQ ID NO: 85 - DNA, 18 bp, Artificial
  Targeting sequence
tataaagtcctagaatgt

SEQ ID NO: 86 - DNA, 19 bp, Artificial
  Targeting sequence
aacagtttgcattcatgga

SEQ ID NO: 87 - DNA, 18 bp, Artificial
  Targeting sequence
tggccatctctgacctgt

SEQ ID NO: 88 - DNA, 18 bp, Artificial
  Targeting sequence
tagtgagcccagaagggg

SEQ ID NO: 89 - DNA, 19 bp, Artificial
  Targeting sequence
ccagaaggggacagtaaga

SEQ ID NO: 90 - DNA, 18 bp, Artificial
  Targeting sequence
taggtacctggctgtcgt

SEQ ID NO: 91 - DNA, 18 bp, Artificial
  Targeting sequence
tgaccgtcctggctttta

SEQ ID NO: 92 - DNA, 19 bp, Artificial
  Targeting sequence
ctgacaatcgataggtacc

SEQ ID NO: 93 - DNA, 18 bp, Artificial
  Targeting sequence
tgtcatggtcatctgcta

SEQ ID NO: 94 - DNA, 18 bp, Artificial
  Targeting sequence
tcgacaccgaagcagagt

SEQ ID NO: 95 - DNA, 19 bp, Artificial
  Targeting sequence
acaccgaagcagagttttt

SEQ ID NO: 96 - DNA, 18 bp, Artificial
  Targeting sequence
tgcccccgcgaggccaca

SEQ ID NO: 97 - DNA, 18 bp, Artificial
  Targeting sequence
tctggaagttgaacaccc

SEQ ID NO: 98 - DNA, 19 bp, Artificial
  Targeting sequence
ggaagttgaacacccttgc

SEQ ID NO: 99 - DNA, 90 bp, Artificial
  Target sequence
ctactgtcattcagggcaatacccagacgagaaagctgagggtataacaggtttcaagcttggcagtctgactacagaggccactggctt

SEQ ID NO: 100 - DNA, 90 bp, Artificial
  Target sequence
ctactgtcattcagcccaataccctaacgagaaagctgagggtataacaggtttcaagcttggcagtctgactacagaggccactggctt

SEQ ID NO: 101 - DNA, 90 bp, Artificial
  Target sequence
ctactgtcattcagcccaatacccagacgagaaaagtgagggtataacaggtttcaagcttggcagtctgactacagaggccactggctt

SEQ ID NO: 102 - DNA, 90 bp, Artificial
  Target sequence
ctactgtcattcagcccaatacccagacgagaaagctgagggtataacaggtttcaagcttggcagtctgactacagaggccactggctt

SEQ ID NO: 103 - DNA, 90 bp, Artificial
  Target sequence
ctactgtcattcagcccaatacccagacgagaaagctgagggtataacaggtttgtagcttggcagtctgactacagaggccactggctt

SEQ ID NO: 104 - DNA, 90 bp, Artificial
  Target sequence
ctactgtcattcagcccaatacccagacgagaaagctgagggtataacaggtttcaagcttggctctctgactacagaggccactggctt

SEQ ID NO: 105 - DNA, 90 bp, Artificial
  Target sequence
ctactgtcattcagcccaatacccagacgagaaagctgagggtataacaggtttcaagcttggcagtctgactagtgaggccactggctt

SEQ ID NO: 106 - DNA, 90 bp, Artificial
  Target sequence
cactttatatttccctgcttaaacagtcccccgagggtgggtgcggaaaaggctctacacttgttatcattccctctccaccacaggcat

SEQ ID NO: 107 - DNA, 90 bp, Artificial
  Target sequence
tttgtatttgggtttttttaaaacctccactctacagttaagaattctaaggcacagagcttcaataatttggtcagagccaagtagcag

SEQ ID NO: 108 - DNA, 90 bp, Artificial
  Target sequence
ggaggttaaacccagcagcatgactgcagttcttaatcaatgccccttgaattgcacatatgggatgaactagaacattttctcgatgat

SEQ ID NO: 109 - DNA, 90 bp, Artificial
  Target sequence
ctcgatgattcgctgtccttgttatgattatgttactgagctctactgtagcacagacatatgtccctatatggggcgggggtgggggtg

SEQ ID NO: 110 - DNA, 90 bp, Artificial
  Taregt sequence
ggtgtcttgatcgctgggctatttctatactgttctggcttttcggaagcagtcatttctttctattctccaagcaccagcaattagctt

SEQ ID NO: 111 - DNA, 90 bp, Artificial
  Target sequence
gcttctagtttgctgaaactaatctgctatagacagagactccgacgaaccaattttattaggatttgatcaaataaactctctctgaca

SEQ ID NO: 112 - DNA, 90 bp, Artificial
  Target sequence
gaaagagtaactaagagtttgatgtttactgagtgcatagtatgcactagatgctggccgtggatgcctcatagaatcctcccaacaact

SEQ ID NO: 113 - DNA, 90 bp, Artificial
  Target sequence
gctagatgctggccgtggatgcctcatagaatcctcccaacaaccgatgaaatgactactgtcattcagcccaatacccagacgagaaag

SEQ ID NO: 114 - DNA, 90 bp, Artificial
  Target sequence
acaggtttcaagcttggcagtctgactacagaggccactggctttacccctgggttagtctgcctctgtaggattgggggcacgtaattt

SEQ ID NO: 115 - DNA, 90 bp, Artificial
  Target sequence
ttagtctgcctctgtaggattgggggcacgtaattttgctgtttaaggtctcatttgccttcttagagatcacaagccaaagctttttat

SEQ ID NO: 116 - DNA, 90 bp, Artificial
  Target sequence
ggaagcccagagggcatcttgtggctcgggagtagctctctgctaccttctcagctctgctgacaatacttgagattttcagatgtcacc

SEQ ID NO: 117 - DNA, 90 bp, Artificial
  Target sequence
tcagctctgctgacaatacttgagattttcagatgtcaccaaccagcaagagagcttgatatgactgtatatagtatagtcataaagaac

SEQ ID NO: 118 - DNA, 90 bp, Artificial
  Target sequence
cataaagaacctgaacttgaccatatacttatgtcatgtggaaatcttctcatagcttcagatagattatatctggagtgaagaatcctg

SEQ ID NO: 119 - DNA, 90 bp, Artificial
  Target sequence
gtggaaaatttctcatagcttcagatagattatatctggagtgagcaatcctgccacctatgtatctggcatagtgtgagtcctcataaa

SEQ ID NO: 120 - DNA, 90 bp, Artificial
  Target sequence
ggtttgaagggcaacaaaatagtgaacagagtgaaaatccccacctagatcctgggtccagaaaaagatgggaaacctgtttagctcacc

SEQ ID NO: 121 - DNA, 30 bp, Artificial
  Target sequence
ggccactagggacaaaattggtgacagaaa

SEQ ID NO: 122 - DNA, 50 bp, Artificial
  Target sequence
cccacagtggggccactagggacaaaattggtgacagaaaagccccatcc

SEQ ID NO: 123 - DNA, 70 bp, Artificial
  Target sequence
tcccctccaccccacagtggggccactagggacaaaattggtgacagaaaagccccatccttaggcctcc

SEQ ID NO: 124 - DNA, 90 bp, Artificial
  Target sequence
cttttatctgtcccctccaccccacagtggggccactagggacaaaattggtgacagaaaagccccatccttaggcctcctccttcctag

SEQ ID NO: 125 - DNA, 110 bp, Artificial
  Target sequence
gttctgggtacttttatctgtcccctccaccccacagtggggccactagggacaaaattggtgacagaaaagccccatccttaggcctcctccttcctagtctcctgata

SEQ ID NO: 126 - DNA, 30 bp, Artificial
  Target sequence
tttctgtcaccaatggtgtccctagtggcc

SEQ ID NO: 127 - DNA, 50 bp, Artificial
  Target sequence
ggatggggcttttctgtcaccaatggtgtccctagtggccccactgtggg

SEQ ID NO: 128 - DNA, 70 bp, Artificial
  Target sequence
ggaggcctaaggatggggcttttctgtcaccaatggtgtccctagtggccccactgtggggtggagggga

SEQ ID NO: 129 - DNA, 90 bp, Artificial
  Target sequence
ctaggaaggaggaggcctaaggatggggcttttctgtcaccaatggtgtccctagtggccccactgtggggtggaggggacagataaaag

SEQ ID NO: 130 - DNA, 110 bp, Artificial
  Target sequence
tatcaggagactaggaaggaggaggcctaaggatggggcttttctgtcaccaatggtgtccctagtggccccactgtggggtggaggggacagataaaagtacccagaac

SEQ ID NO: 131 - DNA, 70 bp, Artificial
  Target sequence
ttctagtaaccactcaggacaggggggttcagcccaaaaattcacaagaaagtggggacccatgggaaat

SEQ ID NO: 132 - DNA, 70 bp, Artificial
  Target sequence
cagcaagtcagcagcacagcgtgtgtgactccgagggtgctccgctagcccacattgccctctgggggtg

SEQ ID NO: 133 - DNA, 70 bp, Artificial
  Target sequence
gtcagactgccaagcttgaaacctgtcttaccctctactttctcgtctgggtattgggctgaatgacagt

SEQ ID NO: 134 - DNA, 70 bp, Artificial
  Target sequence
cagagctgagaagacagcagagagctactcccgaagcacaagatgccctctgggcttccgtgaccttggc

SEQ ID NO: 135 - DNA, 70 bp, Artificial
  Target sequence
ctgacaatacttgagattttcagatgtcaccaacgaccaagagagcttgatatgactgtatatagtatag

SEQ ID NO: 136 - DNA, 70 bp, Artificial
  Target sequence
cagatacataggtggcaggattcttcactccagacttaatctatctgaagctatgagaaattttccacat

SEQ ID NO: 137 - DNA, 70 bp, Artificial
  Target sequence
tatatgattgatttgcacagctcatctggccagataagctgagacatccgttcccctacaagaaactctc

SEQ ID NO: 138 - DNA, 70 bp, Artificial
  Target sequence
atctggccagaagagctgagacatccgttccccttgaagaaactctccccggtaagtaacctctcagctg

SEQ ID NO: 139 - DNA, 70 bp, Artificial
  Target sequence
aggcatctcactggagagggtttagttctccttaagagaagataagatttcaagagggaagctaagactc

SEQ ID NO: 140 - DNA, 70 bp, Artificial
  Target sequence
ataatataataaaaaatgtttcgtctgccaccactaatgaatgtcatgcattctgggtagtttagtctta

SEQ ID NO: 141 - DNA, 70 bp, Artificial
  Target sequence
tttataaagtcctagaatgtatttagttgccctcgttgaatgcaaactgttttatacatcaataggtttt

SEQ ID NO: 142 - DNA, 70 bp, Artificial
  Target sequence
gctcaacctggccatctctgacctgtttttccttcccactgtccccttctgggctcactatgctgccgcc

SEQ ID NO: 143 - DNA, 70 bp, Artificial
  Target sequence
ttttaaagcaaacacagcatggacgacagccaggctcctatcgattgtcaggaggatgatgaagaagatt

SEQ ID NO: 144 - DNA, 70 bp, Artificial
  Target sequence
gcttgtcatggtcatctgctactcgggaatcctaattactctgcttcggtgtcgaaatgagaagaagagg

SEQ ID NO: 145 - DNA, 70 bp, Artificial
  Target sequence
atactgcccccgcgaggccacattggcaaaccagcttgggtgttcaacttccagacttggccatggagaa

SEQ ID NO: 146 - DNA, 90 bp, Artificial
  Target sequence
ctgaagaatttcccatgggtccccactttcttgtgaatccttggagtgaacccccctgtcctgagtggttactagaacacacctctggac

SEQ ID NO: 147 - DNA, 90 bp, Artificial
  Target sequence
tggaagtatcttgccgaggtcacacagcaagtcagcagcacagccagtgtgactccgagcctgctccgctagcccacattgccctctggg

SEQ ID NO: 148 - DNA, 90 bp, Artificial; identical to SEQ ID NO: 102
  Target sequence

SEQ ID NO: 149 - DNA, 90 bp, Artificial; identical to SEQ ID NO: 116
  Target sequence

SEQ ID NO: 150 - DNA, 90 bp, Artificial
  Target sequence
tcagctctgctgacaatacttgagattttcagatgtcaccaacgcccaagagagcttgatatgactgtatatagtatagtcataaagaac

SEQ ID NO: 151 - DNA, 90 bp, Artificial; identical to SEQ ID NO: 119
  Target sequence

SEQ ID NO: 152 - DNA, 90 bp, Artificial
  Target sequence
gaaacagcatttcctacttttatactgtctatatgattgatttggtcagctcatctggccagaagagctgagacatccgttcccctacaa

SEQ ID NO: 153 - DNA, 90 bp, Artificial
  Target sequence
ttgatttgcacagctcatctggccagaagagctgagacatccgtatccctacaagaaactctccccggtaagtaacctctcagctgcttg

SEQ ID NO: 154 - DNA, 90 bp, Artificial
  Target sequence
ggagagggtttagttctccttagcagaagataagatttcaagatgagagctaagactcatctctctgcaaatctttcttttgagaggtaa

SEQ ID NO: 155 - DNA, 90 bp, Artificial
  Target sequence
taatataataaaaaatgtttcgtctgccaccacagatgaatgtcgagcattctgggtagtttagtcttataaccagctgtcttgcctagt

SEQ ID NO: 156 - DNA, 90 bp, Artificial
  Target sequence
ttaaaaacctattgatgtataaaacagtttgcattcatggagggtgactaaatacattctaggactttataaaagatcactttttattta

SEQ ID NO: 157 - DNA, 90 bp, Artificial
  Target sequence
gacatctacctgctcaacctggccatctctgacctgtttttcctatttactgtccccttctgggctcactatgctgccgcccagtgggac

SEQ ID NO: 158 - DNA, 90 bp, Artificial
  Target sequence
tcatcctcctgacaatcgataggtacctggctgtcgtccatgctacgtttgctttaaaagccaggacggtcacctttggggtggtgacaa

SEQ ID NO: 159 - DNA, 90 bp, Artificial
  Target sequence
ggctggtcctgccgctgcttgtcatggtcatctgctactcgggagacctaaaaactctgcttcggtgtcgaaatgagaagaagaggcaca

SEQ ID NO: 160 - DNA, 90 bp, Artificial
  Target sequence
ggcaagccttgggtcatactgcccccgcgaggccacattggcaagtcagcaagggtgttcaacttccagacttggccatggagaagacat

SEQ ID NO: 161 - DNA, 59 bp, Artificial
  PCR primer
acactctttccctacacgacgctcttccgatctcgtgattttgcagtgtgcgttactcc

SEQ ID NO: 162 - DNA, 59 bp, Artificial
  PCR primer
acactctttccctacacgacgctcttccgatctacatcgtttgcagtgtgcgttactcc

SEQ ID NO: 163 - DNA, 59 bp, Artificial
  PCR primer
acactctttccctacacgacgctcttccgatctgcctaatttgcagtgtgcgttactcc

SEQ ID NO: 164 - DNA, 59 bp, Artificial
  PCR primer
acactctttccctacacgacgctcttccgatcttggtcatttgcagtgtgcgttactcc

SEQ ID NO: 165 - DNA, 54 bp, Artificial
  PCR primer
ctcggcattcctgctgaaccgctcttccgatctccaagcaactaagtcacagca

SEQ ID NO: 166 - DNA, 58 bp, Artificial
  PCR primer
acactctttccctacacgacgctcttccgatctcgtgatatgaggaaatggaagcttg

SEQ ID NO: 167 - DNA, 58 bp, Artificial
  PCR primer
acactctttccctacacgacgctcttccgatctacatcgatgaggaaatggaagcttg

SEQ ID NO: 168 - DNA, 58 bp, Artificial
  PCR primer
acactctttccctacacgacgctcttccgatctgcctaaatgaggaaatggaagcttg

SEQ ID NO: 169 - DNA, 58 bp, Artificial
  PCR primer
acactctttccctacacgacgctcttccgatcttggtcaatgaggaaatggaagcttg

SEQ ID NO: 170 - DNA, 51 bp, Artificial
  PCR primer
ctcggcattcctgctgaaccgctcttccgatctcattagggtattggagga

SEQ ID NO: 171 - DNA, 58 bp, Artificial
  PCR primer
acactctttccctacacgacgctcttccgatctcgtgataatcctcccaacaactcat

SEQ ID NO: 172 - DNA, 58 bp, Artificial
  PCR primer
acactctttccctacacgacgctcttccgatctacatcgaatcctcccaacaactcat

SEQ ID NO: 173 - DNA, 58 bp, Artificial
  PCR primer
acactctttccctacacgacgctcttccgatctgcctaaaatcctcccaacaactcat

SEQ ID NO: 174 - DNA, 58 bp, Artificial
  PCR primer
acactctttccctacacgacgctcttccgatcttggtcaaatcctcccaacaactcat

SEQ ID NO: 175 - DNA, 52 bp, Artificial
  PCR primer
ctcggcattcctgctgaaccgctcttccgatctcccaatcctacagaggcag

SEQ ID NO: 176 - DNA, 58 bp, Artificial
  PCR primer
acactctttccctacacgacgctcttccgatctcgtgataagccaaagctttttattc

SEQ ID NO: 177 - DNA, 58 bp, Artificial
  PCR primer
acactctttccctacacgacgctcttccgatctacatcgaagccaaagctttttattc

SEQ ID NO: 178 - DNA, 58 bp, Artificial
  PCR primer
acactctttccctacacgacgctcttccgatctgcctaaaagccaaagctttttattc

SEQ ID NO: 179 - DNA, 58 bp, Artificial
  PCR primer
acactctttccctacacgacgctcttccgatcttggtcaaagccaaagctttttattc

SEQ ID NO: 180 - DNA, 53 bp, Artificial
  PCR primer
acactctttccctacacgacgctcttccgatctaagccaaagctttttattct

SEQ ID NO: 181 - DNA, 59 bp, Artificial
  PCR primer
acactctttccctacacgacgctcttccgatctcgtgatatcttgtggctcgggagtag

SEQ ID NO: 182 - DNA, 59 bp, Artificial
  PCR primer
acactctttccctacacgacgctcttccgatctacatcgatcttgtggctcgggagtag

SEQ ID NO: 183 - DNA, 53 bp, Artificial
  PCR primer
ctcggcattcctgctgaaccgctcttccgatcttggcaggattcttcactcca

SEQ ID NO: 184 - DNA, 59 bp, Artificial
  PCR primer
acactctttccctacacgacgctcttccgatctcgtgatctattttgttgcccttcaaa

SEQ ID NO: 185 - DNA, 59 bp, Artificial
  PCR primer
acactctttccctacacgacgctcttccgatctacatcgctattttgttgcccttcaaa

SEQ ID NO: 186 - DNA, 55 bp, Artificial
  PCR primer
ctcggcattcctgctgaaccgctcttccgatctaacctgaacttgaccatatact

SEQ ID NO: 187 - DNA, 59 bp, Artificial
  PCR primer
acactctttccctacacgacgctcttccgatctcgtgatcagctgagaggttacttacc

SEQ ID NO: 188 - DNA, 59 bp, Artificial
  PCR primer
acactctttccctacacgacgctcttccgatctacatcgcagctgagaggttacttacc

SEQ ID NO: 189 - DNA, 53 bp, Artificial
  PCR primer
ctcggcattcctgctgaaccgctcttccgatctaatgatttaactccaccctc

SEQ ID NO: 190 - DNA, 60 bp, Artificial
  PCR primer
acactctttccctacacgacgctcttccgatctcgtgatactccaccctccttcaaaaga

SEQ ID NO: 191 - DNA, 60 bp, Artificial
  PCR primer
acactctttccctacacgacgctcttccgatctacatcgactccaccctccttcaaaaga

SEQ ID NO: 192 - DNA, 52 bp, Artificial
  PCR primer
ctcggcattcctgctgaaccgctcttccgatcttggtgtttgccaaatgtct

SEQ ID NO: 193 - DNA, 59 bp, Artificial
  PCR primer
acactctttccctacacgacgctcttccgatctcgtgatgggcacatattcagaaggca

SEQ ID NO: 194 - DNA, 59 bp, Artificial
  PCR primer
acactctttccctacacgacgctcttccgatctacatcggggcacatattcagaaggca

SEQ ID NO: 195 - DNA, 56 bp, Artificial
  PCR primer
ctcggcattcctgctgaaccgctcttccgatctagtgaaagactttaaagggagca

SEQ ID NO: 196 - DNA, 59 bp, Artificial
  PCR primer
acactctttccctacacgacgctcttccgatctcgtgatcacaattaagagttgtcata

SEQ ID NO: 197 - DNA, 59 bp, Artificial
  PCR primer
acactctttccctacacgacgctcttccgatctacatcgcacaattaagagttgtcata

SEQ ID NO: 198 - DNA, 53 bp, Artificial
  PCR primer
ctcggcattcctgctgaaccgctcttccgatctctcagctagagcagctgaac

SEQ ID NO: 199 - DNA, 51 bp, Artificial
  PCR primer
ctcggcattcctgctgaaccgctcttccgatctgacacttgataatccatc

SEQ ID NO: 200 - DNA, 60 bp, Artificial
  PCR primer
acactctttccctacacgacgctcttccgatctacatcgtcaatgtagacatctatgtag

SEQ ID NO: 201 - DNA, 60 bp, Artificial
  PCR primer
acactctttccctacacgacgctcttccgatctcgtgattcaatgtagacatctatgtag

SEQ ID NO: 202 - DNA, 59 bp, Artificial
  PCR primer
acactctttccctacacgacgctcttccgatctcgtgatactgcaaaaggctgaagagc

SEQ ID NO: 203 - DNA, 59 bp, Artificial
  PCR primer
acactctttccctacacgacgctcttccgatctacatcgactgcaaaaggctgaagagc

SEQ ID NO: 204 - DNA, 59 bp, Artificial
  PCR primer
acactctttccctacacgacgctcttccgatctgcctaaactgcaaaaggctgaagagc

SEQ ID NO: 205 - DNA, 59 bp, Artificial
  PCR primer
acactctttccctacacgacgctcttccgatcttggtcaactgcaaaaggctgaagagc

SEQ ID NO: 206 - DNA, 57 bp, Artificial
  PCR primer
ctcggcattcctgctgaaccgctcttccgatctgcctataaaatagagccctgtcaa

SEQ ID NO: 207 - DNA, 60 bp, Artificial
  PCR primer
acactctttccctacacgacgctcttccgatctcgtgatctctattttataggcttcttc

SEQ ID NO: 208 - DNA, 60 bp, Artificial
  PCR primer
acactctttccctacacgacgctcttccgatctacatcgctctattttataggcttcttc

SEQ ID NO: 209 - DNA, 52 bp, Artificial
  PCR primer
ctcggcattcctgctgaaccgctcttccgatctagccaccacccaagtgatc

SEQ ID NO: 210 - DNA, 60 bp, Artificial
  PCR primer
acactctttccctacacgacgctcttccgatctacatcgttccagacattaaagatagtc

SEQ ID NO: 211 - DNA, 60 bp, Artificial
  PCR primer
acactctttccctacacgacgctcttccgatctcgtgatttccagacattaaagatagtc

SEQ ID NO: 212 - DNA, 54 bp, Artificial
  PCR primer
ctcggcattcctgctgaaccgctcttccgatctaatcatgatggtgaagataag

SEQ ID NO: 213 - DNA, 60 bp, Artificial
  PCR primer
acactctttccctacacgacgctcttccgatctcgtgatccggcagagacaaacattaaa

SEQ ID NO: 214 - DNA, 54 bp, Artificial
  PCR primer
acactctttccctacacgacgctcttccgatctccggcagagacaaacattaaa

SEQ ID NO: 215 - DNA, 53 bp, Artificial
  PCR primer
ctcggcattcctgctgaaccgctcttccgatctagctaggaagccatggcaag

SEQ ID NO: 216 - DNA, 47 bp, Artificial
  PCR primer
aatgatacggcgaccaccgagatctacactctttccctacacgacgc

SEQ ID NO: 217 - DNA, 50 bp, Artificial
  PCR primer
caagcagaagacggcatacgagatcggtctcggcattcctgctgaaccgc

SEQ ID NO: 218 - DNA, 58 bp, Artificial
  PCR primer
acactctttccctacacgacgctcttccgatctagtgcatagtatgtgctagatgctg

SEQ ID NO: 219 - DNA, 59 bp, Artificial
  PCR primer
gtgactggagttcagacgtgtgctcttccgatcttgatctctaagaaggcaaatgagac

SEQ ID NO: 220 - DNA, 64 bp, Artificial
  PCR primer
  misc_feature (25)..(30): n is a, c, g, or t
caagcagaagacggcatacgagatnnnnnngtgactggagttcagacgtgtgctcttccgatct

SEQ ID NO: 221 - DNA, 58 bp, Artificial
  PCR primer
aatgatacggcgaccaccgagatctacactctttccctacacgacgctcttccgatct

SEQ ID NO: 222 - protein, 34 aa, Artificial
  Deduced TALE template amino acid sequence
  misc_feature (12)..(13): Xaa can be any naturally occurring amino acid
LTPEQVVAIASXXGGKQALETVQRLLPVLCQAHG

SEQ ID NO: 223 - DNA, 246 bp, Artificial
  TALE dimer nucleotide sequence
cgattactgcctgtcttatgtcaggcccatggccttactcctgagcaagtcgtagctatcgccagcaacataggtgggaaacaggccctggaaaccgtacaacgtctcctcccagtactttgtcaagcacacgggttgacaccggaacaagtggtggcgattgcgtcccacgatggaggcaagcaggcactggagaccgtccaacggcttcttccggttctttgccaggctcatgggctcacgcca

SEQ ID NO: 224 - protein, 82 aa, Artificial
  Deduced TALE dimer amino acid sequence
RLLPVLCQAHGLTPEQVVAIASNIGGKQALETVQRLLPVLCQAHGLTPEQVVAIASHDGGKQALETVQRLLPVLCQAHGLTP